European Patent Application EP 4 458 375 A1, published November 6, 2024. Title: Pharmaceutical composition for treating and/or preventing aneurysm, method for assisting diagnosis of aneurysm and method for evaluating aneurysm therapeutic agents. Applicant: 国立研究開発法人理化学研究所. The sequence listing filed with the application follows.

SEQUENCE LISTING (19 sequences)

SEQ ID NO: 1 - DNA, 3321 bp, Homo sapiens
  source 1..3321: mol_type = genomic DNA
atgcggcttccgggtgcgatgccagctctggccctcaaaggcgagctgctgttgctgtctctcctgttacttctggaaccacagatctctcagggcctggtcgtcacacccccggggccagagcttgtcctcaatgtctccagcaccttcgttctgacctgctcgggttcagctccggtggtgtgggaacggatgtcccaggagcccccacaggaaatggccaaggcccaggatggcaccttctccagcgtgctcacactgaccaacctcactgggctagacacgggagaatacttttgcacccacaatgactcccgtggactggagaccgatgagcggaaacggctctacatctttgtgccagatcccaccgtgggcttcctccctaatgatgccgaggaactattcatctttctcacggaaataactgagatcaccattccatgccgagtaacagacccacagctggtggtgacactgcacgagaagaaaggggacgttgcactgcctgtcccctatgatcaccaacgtggcttttctggtatctttgaggacagaagctacatctgcaaaaccaccattggggacagggaggtggattctgatgcctactatgtctacagactccaggtgtcatccatcaacgtctctgtgaacgcagtgcagactgtggtccgccagggtgagaacatcaccctcatgtgcattgtgatcgggaatgaggtggtcaacttcgagtggacatacccccgcaaagaaagtgggcggctggtggagccggtgactgacttcctcttggatatgccttaccacatccgctccatcctgcacatccccagtgccgagttagaagactcggggacctacacctgcaatgtgacggagagtgtgaatgaccatcaggatgaaaaggccatcaacatcaccgtggttgagagcggctacgtgcggctcctgggagaggtgggcacactacaatttgctgagctgcatcggagccggacactgcaggtagtgttcgaggcctacccaccgcccactgtcctgtggttcaaagacaaccgcaccctgggcgactccagcgctggcgaaatcgccctgtccacgcgcaacgtgtcggagacccggtatgtgtcagagctgacactggttcgcgtgaaggtggcagaggctggccactacaccatgcgggccttccatgaggatgctgaggtccagctctccttccagctacagatcaatgtccctgtccgagtgctggagctaagtgagagccaccctgacagtggggaacagacagtccgctgtcgtggccggggcatgccccagccgaacatcatctggtctgcctgcagagacctcaaaaggtgtccacgtgagctgccgcccacgctgctggggaacagttccgaagaggagagccagctggagactaacgtgacgtactgggaggaggagcaggagtttgaggtggtgagcacactgcgtctgcagcacgtggatcggccactgtcggtgcgctgcacgctgcgcaacgctgtgggccaggacacgcaggaggtcatcgtggtgccacactccttgccctttaaggtggtggtgatctcagccatcctggccctggtggtgctcaccatcatctcccttatcatcctcatcatgctttggcagaagaagccacgttacgagatccgatggaaggtgattgagtctgtgagctctgacggccatgagtacatctacgtggaccccatgcagctgccctatgactccacgtgggagctgccgcgggaccagcttgtgctgggacgcaccctcggctctggggcctttgggcaggtggtggaggccacggctcatggcctgagccattctcaggccacgatgaaagtggccgtcaagatgcttaaatccacagcccgcagcagtgagaagcaagcccttatgtcggagctgaagatcatgagtcaccttgggccccacctgaacgtggtcaacctgttgggggcctgcaccaaaggaggacccatctatatcatcactgagtactgccgctacggagacctggtggactacctgcaccgcaacaaacacaccttcctgcagcaccactccgacaagcgccgcccgcccagcgcggagctctacagcaatgctctgcccgttgggctccccctgcccagccatgtgtccttgaccggggagagcgacggtggctacatggacatgagcaaggacgagtcggtggactatgtgcccatgctggacatgaaaggagacgtcaaatatgcagacatcgagtcctccaactacatggccccttacgataactacgttccctctgcccctgagaggacctgccgagcaactttgatcaacgagtctccagtgctaagctacatggacctcgtgggcttcagctaccaggtggccaatggcatggagtttctggcctccaagaactgcgtccacagagacctggcggctaggaacgtgctcatctgtgaaggcaagctggtcaagatctgtgactttggcctggctcgagacatcatgcgggactcgaattacatctccaaaggcagcacctttttgcctttaaagtggatggctccggagagcatcttcaacagcctctacaccaccctgagcgacgtgtggtccttcgggatcctgctctgggagatcttcaccttgggtggcaccccttacccagagctgcccatgaacgagcagttctacaatgccatcaaacggggttaccgcatggcccagcctgcccatgcctccgacgagatctatgagatcatgcagaagtgctgggaagagaagtttgagattcggccccccttctcccagctggtgctgcttctcgagagactgttgggcgaaggttacaaaaagaagtaccagcaggtggatgaggagtttctgaggagtgaccacccagccatccttcggtcccaggcccgcttgcctgggttccatggcctccgatctcccctggacaccagctccgtcctctatactgccgtgcagcccaatgagggtgacaacgactatatcatccccctgcctgaccccaaacccgaggttgctgacgagggcccactggagggttcccccagcctagccagctccaccctgaatgaagtcaacacctcctcaaccatctcctgtgacagccccctggagccccaggacgaaccagagccagagccccagcttgagctccaggtggagccggagccagagctggaacagttgccggattcggggtgccctgcgcctcgggcggaagcagaggatagcttcctgtaa

SEQ ID NO: 2 - protein, 1106 aa, Homo sapiens
MRLPGAMPALALKGELLLLSLLLLLEPQISQGLVVTPPGPELVLNVSSTFVLTCSGSAPVVWERMSQEPPQEMAKAQDGTFSSVLTLTNLTGLDTGEYFCTHNDSRGLETDERKRLYIFVPDPTVGFLPNDAEELFIFLTEITEITIPCRVTDPQLVVTLHEKKGDVALPVPYDHQRGFSGIFEDRSYICKTTIGDREVDSDAYYVYRLQVSSINVSVNAVQTVVRQGENITLMCIVIGNEVVNFEWTYPRKESGRLVEPVTDFLLDMPYHIRSILHIPSAELEDSGTYTCNVTESVNDHQDEKAINITVVESGYVRLLGEVGTLQFAELHRSRTLQVVFEAYPPPTVLWFKDNRTLGDSSAGEIALSTRNVSETRYVSELTLVRVKVAEAGHYTMRAFHEDAEVQLSFQLQINVPVRVLELSESHPDSGEQTVRCRGRGMPQPNIIWSACRDLKRCPRELPPTLLGNSSEEESQLETNVTYWEEEQEFEVVSTLRLQHVDRPLSVRCTLRNAVGQDTQEVIVVPHSLPFKVVVISAILALVVLTIISLIILIMLWQKKPRYEIRWKVIESVSSDGHEYIYVDPMQLPYDSTWELPRDQLVLGRTLGSGAFGQVVEATAHGLSHSQATMKVAVKMLKSTARSSEKQALMSELKIMSHLGPHLNVVNLLGACTKGGPIYIITEYCRYGDLVDYLHRNKHTFLQHHSDKRRPPSAELYSNALPVGLPLPSHVSLTGESDGGYMDMSKDESVDYVPMLDMKGDVKYADIESSNYMAPYDNYVPSAPERTCRATLINESPVLSYMDLVGFSYQVANGMEFLASKNCVHRDLAARNVLICEGKLVKICDFGLARDIMRDSNYISKGSTFLPLKWMAPESIFNSLYTTLSDVWSFGILLWEIFTLGGTPYPELPMNEQFYNAIKRGYRMAQPAHASDEIYEIMQKCWEEKFEIRPPFSQLVLLLERLLGEGYKKKYQQVDEEFLRSDHPAILRSQARLPGFHGLRSPLDTSSVLYTAVQPNEGDNDYIIPLPDPKPEVADEGPLEGSPSLASSTLNEVNTSSTISCDSPLEPQDEPEPEPQLELQVEPEPELEQLPDSGCPAPRAEAEDSFL

SEQ ID NO: 3 - DNA, 25 bp, synthetic construct
  misc_feature 1..25: note = primer
  source 1..25: mol_type = other DNA
gcagaaggagatccgatggaaggtg

SEQ ID NO: 4 - DNA, 26 bp, synthetic construct
  misc_feature 1..26: note = primer
  source 1..26: mol_type = other DNA
cggatctccttctgccaaagcatgat

SEQ ID NO: 5 - DNA, 25 bp, synthetic construct
  misc_feature 1..25: note = primer
  source 1..25: mol_type = other DNA
acgttaccgatggaaggtgattgag

SEQ ID NO: 6 - DNA, 26 bp, synthetic construct
  misc_feature 1..26: note = primer
  source 1..26: mol_type = other DNA
ttccatcggtaacgtggcttcttctg

SEQ ID NO: 7 - DNA, 26 bp, synthetic construct
  misc_feature 1..26: note = primer
  source 1..26: mol_type = other DNA
gccacgtaacgagatccgatggaagg

SEQ ID NO: 8 - DNA, 26 bp, synthetic construct
  misc_feature 1..26: note = primer
  source 1..26: mol_type = other DNA
atctcgttacgtggcttcttctgcca

SEQ ID NO: 9 - DNA, 26 bp, synthetic construct
  misc_feature 1..26: note = primer
  source 1..26: mol_type = other DNA
ccacgttccgagatccgatggaaggt

SEQ ID NO: 10 - DNA, 26 bp, synthetic construct
  misc_feature 1..26: note = primer
  source 1..26: mol_type = other DNA
gatctcggaacgtggcttcttctgcc

SEQ ID NO: 11 - DNA, 26 bp, synthetic construct
  misc_feature 1..26: note = primer
  source 1..26: mol_type = other DNA
ccacgttgcgagatccgatggaaggt

SEQ ID NO: 12 - DNA, 26 bp, synthetic construct
  misc_feature 1..26: note = primer
  source 1..26: mol_type = other DNA
gatctcgcaacgtggcttcttctgcc

SEQ ID NO: 13 - DNA, 26 bp, synthetic construct
  misc_feature 1..26: note = primer
  source 1..26: mol_type = other DNA
gccacgtgacgagatccgatggaagg

SEQ ID NO: 14 - DNA, 26 bp, synthetic construct
  misc_feature 1..26: note = primer
  source 1..26: mol_type = other DNA
atctcgtcacgtggcttcttctgcca

SEQ ID NO: 15 - DNA, 17670 bp, Homo sapiens
  source 1..17670: mol_type = genomic DNA
atggagaaggaggagacaacccgggagctgctgctgcccaactggcagggtagtggctcccacgggctgaccatcgcccagagggacgacggcgtctttgtgcaggaggtgacgcagaactcccctgcggcccgcactggggtggtcaaggagggggaccagattgtgggtgccaccatctactttgacaacctgcagtcgggtgaggtgacccagctgctgaacaccatggggcaccacacggtgggcctgaagctgcaccgcaagggggaccgctctcccgagcctggccagacctggacccgtgaagtcttcagctcctgcagctctgaagtggttctgagcggggatgatgaggagtaccagcgcatctacaccacgaagatcaagccacggctgaagtcggaagatggagtggaaggagacctcggggagacccagagccgtaccatcacagtgaccagaagggtcacggcctacactgtggatgtgactggccgggaaggagccaaggacatagacatcagtagccctgaattcaagatcaagattccaagacatgaactgactgaaatctccaatgtggatgtggagacccagtctgggaagaccgtgatcagactgccctcgggctcgggggcagcctctccgacaggctctgctgtggatatccgagcaggggccatttctgcttcaggaccagagctccaaggtgctggccactcgaagctccaggtcaccatgcctgggataaaggtgggaggctcaggtgtcaatgtcaatgcaaagggcttggacttgggtggcagaggaggggtccaagttccagcagtggacatttcatcttctcttgggggtagggcagtagaggtacagggcccatctctggagagtggtgatcatggcaaaattaaatttcccaccatgaaagtgccgaaatttggtgtctcaacagggcgtgagggccagacaccaaaggcagggctgagggtttctgcacctgaagtctctgtggggcacaagggcggcaagccaggcttgactatccaagcccctcagctggaagtcagtgtgccctctgccaatattgagggccttgaggggaagctgaagggcccccaaatcactgggccatcacttgagggtgacctaggcctgaaaggtgccaagccacaggggcacattggggtggatgcctctgctccccaaattgggggtagcatcactggccccagtgtggaagttcaggcccctgacattgatgttcaggggcctgggagcaaactgaatgtgcccaagatgaaagtccccaagttctctgtatcaggtgcaaagggagaggaaactgggattgatgtgacactgcctacaggtgaagtgactgttcctggggtctctggggatgtcagcctgcctgagattgctactggtgggctggaaggaaagatgaaaggtactaaagtgaagactcctgaaatgattattcagaaacctaaaatctccatgcaggatgtggatctgagccttgggtctcctaaactgaaaggagatattaaggtttctgctcctggggtgcaaggtgatgttaaaggccctcaagtggcacttaaaggctccagagtggacatagagacaccaaacctagagggaaccttgacaggccctaggcttggcagtccttccgggaaaaccggaacctgtaggatctctatgtcagaagtagacttaaatgtggccgcacctaaagtgaaagggggtgtagatgtcacactccccagagtagaagggaaagtcaaagtccctgaagttgatgtcagaggccccaaagtggatgtcagtgccccagatgtcgaagcgcatggcccagaatggaacctgaaaatgcccaagatgaaaatgcccacgttcagcactccaggagccaaaggggaaggtccagatgttcatatgactctacccaaaggagatatcagtatttcagggcccaaggtcaatgtggaagccccagatgtcaacttggagggtctggggggaaaacttaaaggccccgatgttaagctgcctgatatgagtgtcaagacaccaaagatctccatgcctgatgtagatttgcacgtgaaaggtacaaaggtgaagggagagtatgatgtaactgtaccaaagctggaaggagaactcaaaggcccaaaagtggacattgatgccccagatgtggatgttcatggcccagactggcacttgaagatgcccaagatgaaaatgcccaaattcagtgtgccagggttcaaagcagagggcccagaagtggatgtgaacctgcccaaggctgatgtggacatttccgggcccaagatagatgttactgctcctgatgtgagcattgaggaaccagaagggaaattgaaagggcccaagtttaagatgcctgagatgaacatcaaagtccccaagatctccatgcctgatgtggacttacatctgaaaggccctaacgtaaagggagaatatgatgtcacaatgccaaaggttgaaagtgagattaaagttcctgatgttgaacttaaaagtgccaaaatggacattgatgtcccagatgtggaggttcaaggcccagactggcacctgaagatgcccaagatgaaaatgcccaagttcagcatgcctggcttcaaagcagagggcccagaagtggatgtgaacctgcccaaggctgatgtggacatctcaggacccaaggtgggtgttgaagttccagatgtgaatattgaaggacctgaaggaaagctgaagggccccaagttcaagatgccagagatgaatatcaaggcccccaagatctccatgcctgatgtggacttgcatatgaaaggtcctaaagtaaagggagaatatgatatgacagtgccaaagctggaaggggacctgaaaggcccaaaagtagatgtcagtgccccagatgttgaaatgcagggtcctgactggaacttgaagatgccaaagattaaaatgcccaaatttagcatgcccagcctcaaaggagaggggccagaatttgatgtgaacctgtccaaagcgaatgtggacatttctgcaccaaaagtagatactaatgctccagatctgagccttgaaggacctgaagggaagttgaaaggcccgaagtttaagatgcctgagatgcacttcagagctcctaagatgtctttgccagatgttgacctggatcttaaaggacccaaaatgaaaggaaatgtagatatctctgcaccaaagatagagggtgaaatgcaggttccagatgtggacatcagaggtcccaaggtagatattaaagcaccagatgtggaaggccaaggcctggactggagcctgaaaatacccaagatgaaaatgcccaagttcagcatgcccagcctcaaaggcgagggcccagaagtggatgtgaacttgcctaaggctgacgttgttgtctcaggacccaaggtggacatcgaagccccagatgtgagcctcgaaggtccagaagggaagctgaagggtcccaagtttaagatgcctgagatgcatttcaagacccccaagatctccatgcctgatgtggacttacacttgaaaggccccaaagtcaaaggggatgtggatgtgtctgtgcccaaggtagaaggtgaaatgaaagtgccagatgttgaaatcaaaggacccaaaatggacattgatgccccagatgtggaggttcaaggcccagactggcacctgaagatgcccaagatgaaaatgcccaagtttagcatgcctggcttcaaaggagagggccgagaagtggatgtgaacctgcccaaggctgacattgatgtctcaggacccaaggtggatgttgaagtcccagatgtgagccttgagggcccggaaggaaagctgaagggccccaagtttaagatgcctgagatgcacttcaaggcccccaagatctccatgcctgatgtggacctgaatcttaaggggccaaaattgaagggagatgtggatgtgtccttgcctgaggtagaaggtgaaatgaaagtgccagatgttgacattaaagggcccaaagttgacattagtgctccagatgtggatgttcatggcccagattggcacctgaagatgcccaaggtgaaaatgcccaagttcagcatgcccggcttcaaaggagagggccctgaagtggatgtgaagctgcccaaagctgacgttgatgtctcaggacccaaaatggatgctgaagttccagatgtgaatattgaaggtccagacgcaaaactaaaaggtcccaaattcaagatgccagaaatgagtataaagcctcagaagatatccataccagatgttggtttgcatttgaaaggtcctaaaatgaaaggagattatgatgtaacagttccaaaagtagaaggagagataaaagctcctgatgttgacatcaaaggccccaaagttgatattaatgcaccagatgtggaggttcatggcccagactggcacctgaagatgcccaaggtaaaaatgcccaagttcagcatgcctggctttaaaggagagggcccagaggtggatatgaacctgcccaaggctgaccttggtgtttcaggacccaaggtggacattgatgttccagatgtgaatcttgaagctccagaggggaaactaaaaggccctaagttcaagatgccaagcatgaatatacagacgcacaaaatctctatgcctgatgttggacttaatttgaaagcccctaaactgaaaactgatgtagatgtttcccttcccaaagtggaaggagacttgaagggtcctgaaattgatgtgaaagcccctaagatggatgtgaatgttggtgatattgatattgaaggtccagaagggaagttgaagggccccaagtttaagatgcctgagatgcatttcaaggcccccaagatctccatgcccgatgtggacttacacttgaaaggccccaaagtcaaaggggatatggatgtgtctgtgcccaaggtagaaggtgaaatgaaagtgccagatgttgacattaaagggcccaaagtggacattgatgccccagatgtggaggttcacgacccagattggcacctgaaaatgcccaagatgaaaatgcccaagttcagtatgcctggcttcaaagcagagggccctgaagtggatgtgaatctgccaaaggctgacattgatgtgtctggacccagtgtggacactgatgctcctgatttggatattgagggaccagaaggaaagttgaaaggctccaaatttaagatgcccaagttgaatataaaagctcccaaggtctccatgccagatgtggacttgaatttgaagggacccaaactgaagggagagatagatgcttctgtgccagaactggaaggtgatctcagagggccgcaagttgatgtcaaaggtccttttgtggaagcggaggtgcccgatgttgatctggagtgtcctgatgcaaagttgaaagggcccaagtttaagatgcctgagatgcacttcaaggcccccaagatctccatgcctgatgtggacttacacctgaaaggccccaaagtcaaaggggatgcggatgtgtcggtgccaaaattggagggagatttaacaggccccagtgtgggtgtggaggtgcctgatgttgagctggagtgtcctgatgcaaagttgaaaggccctaaatttaagatgccagacatgcacttcaaggcccccaagatctccatgcctgatgtggacttacacttgaaaggccccaaagtcaaaggggatgtggatgtgtcggtgccaaaattggagggagatttaacaggtcccagtgtgggtgtggaggtgcctgatgttgagctggagtgtcctgatgcaaagttgaaagggcccaagtttaagatgcctgagatgcacttcaagacccccaagatctccatgcctgatgtggacttacacctgaaaggccccaaagtcaaaggggatatggatgtgtctgtgcccaaggtagaaggtgaaatgaaagtgccagatgttgacatcaaaggacccaaaatggacattgatgccccagatgtggatgttcatggcccagactggcacctgaagatgcccaagatgaaaatgcccaagttcagcatgcctggcttcaaagcagagggcccagaagtggatgtgaacttgcccaaggctgatgttgttgtctcaggacccaaggtggatgttgaagtcccagatgtgagccttgaaggtccagaagggaagctgaagggccccaagcttaagatgcctgagatgcacttcaaggcccccaagatctccatgcctgatgtggacttacacttgaaaggccccaaagtcaaaggggatgtggatgtgtctttgccaaaattggagggagatttaacaggccccagtgtggatgtggaggtgcctgatgttgagctggagtgtcctgatgcaaagttgaaagggcccaagtttaagatgcctgagatgcacttcaagacccccaagatctccatgcctgatgtgaacttaaacttgaaaggccccaaagtcaaaggggatatggatgtgtctgttcccaaggtagaaggtgaaatgaaagtgccagatgttgacatcagagggcccaaagtggacattgatgccccagatgtggatgttcatggcccagactggcacctgaagatgcctaagatgaaaatgcccaagttcagcatgcctggcttcaaaggagagggcccagaagtggatgtgaacttgcccaaggctgacgttgatgtctcaggacccaaggtggatgttgaagtcccagatgtgagccttgaaggtccagaagggaagctgaagggccccaagtttaagatgcctgagatgcacttcaagacccccaagatctccatgcctgatgttgatttcaatttaaagggacccaaaatcaaaggagatgttgatgtttctgccccaaagctggagggagagttaaaaggtccagaattggatgtcaaaggtcccaaattagatgctgacatgccagaagtagctgtggaaggcccaaatggcaagtggaaaactcctaagttcaagatgccagatatgcactttaaagctcccaaaatctctatgccagacctcgatctacacttgaagagccccaaggcaaaaggagaggtggatgtagatgttcccaaattggaaggggaccttaaagggccacatgtggatgtcagtgggccagacattgacattgagggaccagagggcaaattgaaaggccctaagttcaagatgcctgatatgcatttcaaagcccccaatatttctatgcctgatgttgatctaaatctcaaaggacccaaaatcaagggggatgtggatgtgtctgtgcctgaggtagaaggtaaacttgaagtaccagatatgaacatcaggggccccaaagttgatgtaaatgcccccgatgtccaagctccagactggcacctgaagatgcccaagatgaaaatgcccaagttcagcatgcctggcttcaaagcagagggccctgaagtagacgtcaacttgcctaaggctgacgttgacatctcaggacccaaggtggacattgaaggccctgatgttaatattgaaggaccagagggaaagttgaaagggcctaagttaaagatgccagagatgaacatcaaagcccccaagatctccatgcctgactttgatttgcatctgaaaggtcccaaggtgaagggcgatgtggatgtttctctgcccaaagtggaaggtgacctcaagggccccgaagttgacatcaaggggcccaaagtggatattaatgccccagatgtgggtgttcaaggcccagactggcacctgaagatgcccaaggtgaaaatgccaaagttcagcatgcctggcttcaaaggagagggcccagatggggatgtgaagctgcccaaggctgacattgatgtctcaggacccaaagtggacattgaaggccctgatgttaacattgaaggaccagagggaaagttgaaagggcctaagttcaagatgccagagatgaatatcaaagcccccaagatctccatgcctgatattgacttaaacctgaaaggacccaaagtgaagggtgatgtggatgtttcccttcctaaagtggaaggtgacctcaagggcccagaagttgacatcaagggcccaaaagtggacattgacgcacctgatgttgatgttcatggcccagactggcacctaaagatgcccaagataaaaatgcccaagatcagcatgcctggcttcaaaggagaaggtccagatgtggacgtgaacctgcccaaggctgacattgatgtctcaggaccgaaagtggatgttgaatgtcccgatgtgaatatcgaaggacctgaaggaaagtggaaaagtccaaagtttaagatgccagagatgcattttaagactccaaagatatccatgccagatattgacctgaatctcacaggtccaaaaataaaaggagatgtggatgttacaggccctaaggtagagggagatctgaaaggtcctgaagttgacctcaaaggccccaaagtggacattgatgtcccagatgttaatgttcagggtccagactggcacctgaagatgcccaagatgaaaatgcccaagttcagcatgcctggcttcaaagcagagggccctgaagtggatgtgaacctgcccaaggctgacgttgatgtctcaggccccaaagtggacgttgaaggccctgatgttaacattgaaggaccagagggaaagttgaaagggcccaagttcaagatgccagagatgaatatcaaagcccccaagatccccatgcctgactttgatttgcatctgaaaggtcccaaggtgaagggcgatgtggatatttctctgcccaaagtggaaggtgacctcaagggccctgaagttgacatcaggggtccccaagtggacattgatgtcccggatgtgggcgttcaaggcccagactggcacctaaaaatgcccaaagtgaaaatgcccaaattcagcatgcctggcttcaaaggagagggcccagatgtggatgtgaacctgcccaaggctgaccttgatgtctcaggacccaaggtggacattgatgttccagatgtgaatatcgaaggcccagagggaaagttgaaaggtcccaaattcaaaatgcctgagatgaacatcaaagcccccaagatctccatgcctgacattgatcttaacctgaaaggtcccaaagtgaagggtgacatggatgtgtctctgccaaaagtggaaggtgacatgaaagttcctgacgtggatattaaaggccccaaagtggatattaatgccccagatgtggatgttcaaggcccagactggcacctgaagatgcctaaaataaaaatgcccaagatcagcatgcctggcttcaaaggagaaggtccagaagtggacgtgaacctgcccaaggctgaccttgacgtctcaggacccaaggtggacgttgatgttccagatgtgaatattgaaggtccagatgcgaaactgaagggccctaaattcaagatgccagagatgaacatcaaagctcctaaaatatcaatgcctgatttggacctcaatcttaaaggccctaaaatgaaaggagaggtggatgtttcacttgcaaatgtagaaggtgatttgaaaggacctgctcttgacataaaaggcccaaagatagatgtagatgctccagatattgacattcatggcccagatgccaaattaaaaggtccaaaactgaagatgcctgacatgcatgtaaacatgcccaagatctccatgccagaaattgacttgaatttgaaaggctcaaagcttaagggagatgttgatgtctctgggcccaagttggaaggtgacattaaagctcccagtttggatataaagggcccagaagtggacgtttccggtcctaagcttaatatcgaaggcaagtcaaagaaatctcgttttaagcttcccaaatttaatttttcgggctctaaagttcagacacctgaagtggatgtcaaaggtaaaaagccagatattgacataacaggtccaaaagttgatattaatgctcctgatgtcgaggtccaaggaaaagtgaaaggatccaagtttaaaatgcctttcctgagtatttcatctcccaaagtttctatgcctgacgtggagctaaatttgaaaagtcccaaagtcaaaggagacttagatattgcaggtcccaatttagaaggtgactttaaaggccccaaagtggatattaaggcaccagaagtcaatcttaatgcacctgatgtggatgttcatggtccagactggaatctgaaaatgcccaagatgaaaatgcccaaattcagtgtgtctggcttaaaagcagaagggccagatgtagctgtggatctaccaaaaggagacatcaacatagagggcccaagtatgaacattgagggcccagatctcaatgtggaaggtccggagggaggcttgaaaggtcccaaattcaagatgcctgacatgaatatcaaagctcccaagatctccatgcctgacattgacttaaacttgaaaggccccaaggtgaaaggtgatgtggatatttctcttcccaaacttgaaggggatctgaaagggccagaggttgatatcaaaggccctaaagtggacatcaatgccccagatgtggatgttcatggtccagactggcatctgaagatgcccaaagtgaaaatgcccaagttcagcatgcctggcttcaaaggagaaggccctgaagtcgatgttaccctccctaaagctgacattgacatttctggtcccaatgtagacgttgatgttccagacgtgaatattgaaggtccagatgcaaagctgaagggccccaagttcaagatgcctgagatgaacatcaaagcccccaagatctccatgcctgactttgacctgaacttgaagggacccaaaatgaagggtgatgtggttgtgtctttgcccaaagtggaaggtgatctaaaaggccctgaggtggacatcaagggccccaaagtggacattgacactcctgacattaacatcgaaggctcagagggtaaattcaagggacccaaatttaagataccagagatgcacctgaaggctcccaaaatatcgatgcctgacattgatttaaacctgaagggccccaaagtcaagggcgatgtggatgtttctctgcccaaaatggaaggtgacctcaagggtcctgaagttgacatcaagggccccaaagtggacattaatgctccagatgttgatgttcaaggcccagactggcacctgaagatgcccaaggtgaaaatgcccaagttcagcatgcctggcttcaaaggagagggcccagatgtggatgtgaacctgcccaaggctgaccttgatgtctcaggacccaaggtggacattgatgttccagatgtgaatatcgaaggcccagagggaaagttgaaaggtcccaaattcaagatgcctgagatgaacatcaaagcccccaagatctccatgcctgacattgatcttaacctgaaaggacccaaagtgaagggtgatatggatgtgtctctgccaaaagtggaaggtgacatgcaagttcctgacttggatattaaaggccccaaagtggatattaatgccccagatgtggatgttcgaggcccagactggcacctgaagatgcctaagataaaaatgcccaagatcagcatgcctggcttcaaaggagaaggtccagaagtggatgtgaacctgcccaaggctgaccttgacgtctcaggacccaaggtggacgttgatgttccagatgtgaatattgaaggtccagatgcgaaactgaagggccctaaattcaagatgccagagatgaacatcaaagcccccaagatctccatgcctgactttgatttgcatctgaaaggccctaaggtgaaaggagatgtggatgtttctctgcctaagatggaaggtgatctaaaggcccctgaagttgacatcaagggccccaaagtggacattgatgccccagatgtggatgttcatggcccagactggcacctgaagatgcccaaggtgaaaatgcccaaattcagcatgccaggatttaaaggagagggcccagaagtggatgttaatttgcccaaagctgacattgatgtctcaggacccaaagtggacattgacactcctgatattgatattcatggtccagaagggaaactgaagggccccaaatttaaaatgcctgacctgcacctcaaggcaccgaagatctctatgcctgaagttgacctgaatctgaaaggtccaaagatgaagggcgacgtggacgtttctctgcccaaagtggaaggcgacctcaagggccctgaagttgacatcaagggccccaaagtggacattgatgtcccagatgtggacgttcaaggcccagactggcacttaaaaatgcccaaagtgaaaatgcccaagttcagcatgcctggcttcaaaggagagggcccagatgtggatgtgaacctgcccaaggctgaccttgacgtctcaggacccaaggtggacattgatgttcctgatgtgaatatcgaaggtccagatgcgaaactaaagggccctaaattcaagatgcctgagatgaacatcaaagcccccaagatctccatgcctgactttgatttgcatctgaaaggtcccaaggtgaagggtgatgtggatgtttcccttcctaaagtggaaggtgacctcaagggcccagaagttgacatcaagggccccaaagtggacatcgatgcccctgatgtagatgttcatggcccagactggcacctgaagatgcccaaggtgaaaatgcccaaattcagcatgccaggattcaaaggagagggcccagatgtggatgttacccttcctaaggctgacattgagatttctggccccaaagtggacattgatgcccctgatgtcagtatcgaaggtccagatgcaaaactcaagggtccaaagttcaagatgccagagatgaacatcaaggcccccaaaatctccatgcctgacattgactttaacttgaagggtcccaaagtgaaaggtgatgtggatgtctctctgcccaaagtggaaggtgatctcaagggccctgaaattgacataaaaggccccagtttggacattgacacacctgatgtcaatattgaaggtccggaaggaaaattgaaggggcccaaatttaagatgcctgagatgaacatcaaagctcccaaaatctctatgcctgactttgatttgcacctgaaaggtcccaaggtgaagggtgatgtggatgtttcactacctaaggtggaaagtgatctgaaagggccagaggtagacattgaaggtcctgaagggaagctcaaaggtcccaagtttaagatgcctgatgtacatttcaaaagcccacaaatctccatgagtgacattgatttgaatttgaaaggacctaagataaaaggagatatggacatttccgttcctaaactggagggagatctgaaaggtcccaaagtggatgtcaaaggccctaaagtgggcattgacactcctgatattgacattcatggtccagaagggaaactgaagggccccaaatttaaaatgcctgacttacacctcaaggcaccgaagatctctatgcctgaagttgacctgaatctgaaaggtccaaaggtgaagggcgacatggacatttctctgcccaaagtggaaggcgacctcaagggccccgaagttgacatcagggaccccaaagtggacattgatgtcccagatgtggacgttcaaggcccagactggcacctaaaaatgcccaaagtgaaaatgcccaagttcagcatgcctggcttcaaaggagagggcccagatgtggatgtgaacctgcccaaggctgacattgatgtctcaggacccaaagtggacgttgatgttcctgatgtgaatatcgaaggtccagatgcgaaactaaagggccccaagttcaagatgcctgagatgagcatcaaagcccccaagatctccatgcctgatattgacttaaacctgaaaggacccaaagtgaagggcgatgtggatgttacccttcctaaagtggaaggtgacctcaagggcccagaagctgacatcaagggcccaaaagtggacatcaacacccctgatgtggatgttcatggcccagactggcacctgaagatgcccaaggtgaaaatgcccaaattcagcatgcctggcttcaaaggagaaggtccagatgtggatgtgagcctgcccaaggccgacatcgatgtctcgggacccaaggtggacgttgatattccagatgtgaatatcgaaggtccagacgcaaaactgaagggccccaagttcaagatgcctgaaataaatatcaaagctcccaagatctccatacctgatgttgacctggatttgaaaggacccaaagtaaaaggagattttgatgtgtctgtccctaaggttgaagggactttgaaaggcccagaagtagatcttaaaggtccacgtctggatttcgaaggccctgatgccaaactcagtggcccatctttgaagatgccatcgctggagatatctgctcctaaagtaactgctcctgatgttgatttgcatctcaaggcaccaaaaattggattttcaggtccgaagttagaaggtggtgaagtggacctcaagggacccaaagttgaagctccaagcttagatgtacacatggacagcccagatattaacatcgaagggccagatgttaaaatccccaaatttaagaaacccaagtttggatttggggcaaaaagccccaaagctgacatcaagtcaccttcactggatgtcactgttcctgaggcagagctgaaccttgagactcctgaaattagtgttggtggcaagggcaagaaaagtaagtttaaaatgcctaaaattcatatgagtggtcctaagattaaggccaaaaaacagggatttgacctgaatgttcctgggggtgaaattgatgccagcctcaaggctccggatgtagatgtcaacatcgcagggccggatgctgcactcaaagtcgacgtgaaatcgcccaaaaccaagaaaacgatgtttggaaaaatgtacttcccagatgtagagtttgacattaaatcacctaaatttaaagctgaggcccctctccctagccccaaactggagggtgaactccaggcacctgatctggaactttctttgccagcgattcacgtcgaaggtcttgacatcaaggcgaaggctcccaaggtcaagatgccagatgtggacatctcagtgccaaaaatagagggtgacctgaaaggccccaaagtgcaggcaaacttgggtgcacctgacatcaacatcgaaggcctagatgctaaagtcaaaacaccgtccttcggcatttctgcccctcaagtctccatccctgatgtgaatgtaaacttgaaaggaccaaagataaagggtgatgtccccagcgtgggactggaaggaccagatgtagatctgcaaggtccagaagcaaaaattaagttccccaagttttccatgcccaagatcggcatcccaggtgtgaaaatggagggtgggggagccgaggtccatgcccagctaccctctcttgaaggagacttgagaggaccagatgttaagctcgaagggcccgatgtttctctaaaggggccaggagtagacttgccttcagtgaacctctctatgccaaaagtctctgggcctgaccttgatctgaacttgaaaggaccaagtttgaagggagacctggatgcatctgttcccagcatgaaggtgcatgctccagggctcaacctcagtggtgtcggtggcaaaatgcaggtgggaggagacggtgtgaaagtgccagggatcgatgccacaacaaagcttaacgttggggcaccagatgtgacactgaggggaccaagcctgcagggagatctggctgtctctggtgacatcaaatgccctaaagtatccgtaggagctcctgatctaagcttggaggcatccgaaggcagcattaaacttcccaaaatgaagctgccccaatttggcatctctactccggggtccgacttgcacgtcaatgccaaggggccacaggtttctggcgaactgaaggggccaggtgtggatgtgaacctgaaagggcctcggatttcagcaccgaatgtggactttaacttggaaggaccaaaagtgaaagggagccttggggccactggtgagatcaaaggccccactgtcggaggaggtcttccaggcattggtgttcaaggcctagaaggaaacctccagatgcctggaattaagtcctctggatgtgatgtgaacctgccaggcgtgaatgtgaaactcccaactgggcagatttctgggcctgaaatcaaaggtggtctgaaaggttcagaagtaggtttccatggggctgctcctgatatcagtgtgaaggggcctgcctttaatatggcatctcctgagtcagattttggcatcaacttgaagggcccaaaaatcaaaggaggtgcggatgtttcagggggtgtcagtgccccagacatcagccttggtgaagggcatttgagtgttaaaggttccgggggtgagtggaagggaccccaagtctcctctgctctcaacttggacacatctaagtttgctgggggccttcatttctcaggaccaaaggtggaaggaggtgtgaaaggaggtcagattggactccaggctcctgggctgagtgtgtctgggcctcaaggtcacttggaaagtggatctggaaaagtaacattccctaaaatgaagatccccaaatttaccttctctggccgtgagctggttggcagagaaatgggggtggatgttcacttccctaaagcagaggccagcatccaagctggtgctggagacggcgagtgggaagagtctgaagtcaaactgaaaaagtccaagatcaaaatgcccaagtttaatttttccaaacctaaagggaaaggtggtgtcactggctcaccagaagcatcaatttctgggtccaaaggtgacctgaaaagttcaaaggccagcctgggctctctggaaggagaggcagaggccgaagcctcttcaccgaaaggcaaattctccttatttaaaagtaagaagccacggcaccgctcaaattcattcagtgatgaaagagagttctctggaccttccaccccgacggggacgctggagtttgaaggtggggaagtgtctctggaaggtgggaaagttaaagggaaacacgggaagctgaaattcggtacctttggtggattggggtcaaagagcaaaggtcattatgaggtgactgggagcgatgatgagacaggcaagttacaggggagtggggtgtccctggcctctaagaagtcccgactgtcctcctcttctagcaatgacagtgggaataaggttggcatccagcttcccgaggtggagctgtcagtttccacaaagaaagag

SEQ ID NO: 16 - protein, 5890 aa, Homo sapiens
MEKEETTRELLLPNWQGSGSHGLTIAQRDDGVFVQEVTQNSPAARTGVVKEGDQIVGATIYFDNLQSGEVTQLLNTMGHHTVGLKLHRKGDRSPEPGQTWTREVFSSCSSEVVLSGDDEEYQRIYTTKIKPRLKSEDGVEGDLGETQSRTITVTRRVTAYTVDVTGREGAKDIDISSPEFKIKIPRHELTEISNVDVETQSGKTVIRLPSGSGAASPTGSAVDIRAGAISASGPELQGAGHSKLQVTMPGIKVGGSGVNVNAKGLDLGGRGGVQVPAVDISSSLGGRAVEVQGPSLESGDHGKIKFPTMKVPKFGVSTGREGQTPKAGLRVSAPEVSVGHKGGKPGLTIQAPQLEVSVPSANIEGLEGKLKGPQITGPSLEGDLGLKGAKPQGHIGVDASAPQIGGSITGPSVEVQAPDIDVQGPGSKLNVPKMKVPKFSVSGAKGEETGIDVTLPTGEVTVPGVSGDVSLPEIATGGLEGKMKGTKVKTPEMIIQKPKISMQDVDLSLGSPKLKGDIKVSAPGVQGDVKGPQVALKGSRVDIETPNLEGTLTGPRLGSPSGKTGTCRISMSEVDLNVAAPKVKGGVDVTLPRVEGKVKVPEVDVRGPKVDVSAPDVEAHGPEWNLKMPKMKMPTFSTPGAKGEGPDVHMTLPKGDISISGPKVNVEAPDVNLEGLGGKLKGPDVKLPDMSVKTPKISMPDVDLHVKGTKVKGEYDVTVPKLEGELKGPKVDIDAPDVDVHGPDWHLKMPKMKMPKFSVPGFKAEGPEVDVNLPKADVDISGPKIDVTAPDVSIEEPEGKLKGPKFKMPEMNIKVPKISMPDVDLHLKGPNVKGEYDVTMPKVESEIKVPDVELKSAKMDIDVPDVEVQGPDWHLKMPKMKMPKFSMPGFKAEGPEVDVNLPKADVDISGPKVGVEVPDVNIEGPEGKLKGPKFKMPEMNIKAPKISMPDVDLHMKGPKVKGEYDMTVPKLEGDLKGPKVDVSAPDVEMQGPDWNLKMPKIKMPKFSMPSLKGEGPEFDVNLSKANVDISAPKVDTNAPDLSLEGPEGKLKGPKFKMPEMHFRAPKMSLPDVDLDLKGPKMKGNVDISAPKIEGEMQVPDVDIRGPKVDIKAPDVEGQGLDWSLKIPKMKMPKFSMPSLKGEGPEVDVNLPKADVVVSGPKVDIEAPDVSLEGPEGKLKGPKFKMPEMHFKTPKISMPDVDLHLKGPKVKGDVDVSVPKVEGEMKVPDVEIKGPKMDIDAPDVEVQGPDWHLKMPKMKMPKFSMPGFKGEGREVDVNLPKADIDVSGPKVDVEVPDVSLEGPEGKLKGPKFKMPEMHFKAPKISMPDVDLNLKGPKLKGDVDVSLPEVEGEMKVPDVDIKGPKVDISAPDVDVHGPDWHLKMPKVKMPKFSMPGFKGEGPEVDVKLPKADVDVSGPKMDAEVPDVNIEGPDAKLKGPKFKMPEMSIKPQKISIPDVGLHLKGPKMKGDYDVTVPKVEGEIKAPDVDIKGPKVDINAPDVEVHGPDWHLKMPKVKMPKFSMPGFKGEGPEVDMNLPKADLGVSGPKVDIDVPDVNLEAPEGKLKGPKFKMPSMNIQTHKISMPDVGLNLKAPKLKTDVDVSLPKVEGDLKGPEIDVKAPKMDVNVGDIDIEGPEGKLKGPKFKMPEMHFKAPKISMPDVDLHLKGPKVKGDMDVSVPKVEGEMKVPDVDIKGPKVDIDAPDVEVHDPDWHLKMPKMKMPKFSMPGFKAEGPEVDVNLPKADIDVSGPSVDTDAPDLDIEGPEGKLKGSKFKMPKLNIKAPKVSMPDVDLNLKGPKLKGEIDASVPELEGDLRGPQVDVKGPFVEAEVPDVDLECPDAKLKGPKFKMPEMHFKAPKISMPDVDLHLKGPKVKGDADVSVPKLEGDLTGPSVGVEVPDVELECPDAKLKGPKFKMPDMHFKAPKISMPDVDLHLKGPKVKGDVDVSVPKLEGDLTGPSVGVEVPDVELECPDAKLKGPKFKMPEMHFKTPKISMPDVDLHLKGPKVKGDMDVSVPKVEGEMKVPDVDIKGPKMDIDAPDVDVHGPDWHLKMPKMKMPKFSMPGFKAEGPEVDVNLPKADVVVSGPKVDVEVPDVSLEGPEGKLKGPKLKMPEMHFKAPKISMPDVDLHLKGPKVKGDVDVSLPKLEGDLTGPSVDVEVPDVELECPDAKLKGPKFKMPEMHFKTPKISMPDVNLNLKGPKVKGDMDVSVPKVEGEMKVPDVDIRGPKVDIDAPDVDVHGPDWHLKMPKMKMPKFSMPGFKGEGPEVDVNLPKADVDVSGPKVDVEVPDVSLEGPEGKLKGPKFKMPEMHFKTPKISMPDVDFNLKGPKIKGDVDVSAPKLEGELKGPELDVKGPKLDADMPEVAVEGPNGKWKTPKFKMPDMHFKAPKISMPDLDLHLKSPKAKGEVDVDVPKLEGDLKGPHVDVSGPDIDIEGPEGKLKGPKFKMPDMHFKAPNISMPDVDLNLKGPKIKGDVDVSVPEVEGKLEVPDMNIRGPKVDVNAPDVQAPDWHLKMPKMKMPKFSMPGFKAEGPEVDVNLPKADVDISGPKVDIEGPDVNIEGPEGKLKGPKLKMPEMNIKAPKISMPDFDLHLKGPKVKGDVDVSLPKVEGDLKGPEVDIKGPKVDINAPDVGVQGPDWHLKMPKVKMPKFSMPGFKGEGPDGDVKLPKADIDVSGPKVDIEGPDVNIEGPEGKLKGPKFKMPEMNIKAPKISMPDIDLNLKGPKVKGDVDVSLPKVEGDLKGPEVDIKGPKVDIDAPDVDVHGPDWHLKMPKIKMPKISMPGFKGEGPDVDVNLPKADIDVSGPKVDVECPDVNIEGPEGKWKSPKFKMPEMHFKTPKISMPDIDLNLTGPKIKGDVDVTGPKVEGDLKGPEVDLKGPKVDIDVPDVNVQGPDWHLKMPKMKMPKFSMPGFKAEGPEVDVNLPKADVDVSGPKVDVEGPDVNIEGPEGKLKGPKFKMPEMNIKAPKIPMPDFDLHLKGPKVKGDVDISLPKVEGDLKGPEVDIRGPQVDIDVPDVGVQGPDWHLKMPKVKMPKFSMPGFKGEGPDVDVNLPKADLDVSGPKVDIDVPDVNIEGPEGKLKGPKFKMPEMNIKAPKISMPDIDLNLKGPKVKGDMDVSLPKVEGDMKVPDVDIKGPKVDINAPDVDVQGPDWHLKMPKIKMPKISMPGFKGEGPEVDVNLPKADLDVSGPKVDVDVPDVNIEGPDAKLKGPKFKMPEMNIKAPKISMPDLDLNLKGPKMKGEVDVSLANVEGDLKGPALDIKGPKIDVDAPDIDIHGPDAKLKGPKLKMPDMHVNMPKISMPEIDLNLKGSKLKGDVDVSGPKLEGDIKAPSLDIKGPEVDVSGPKLNIEGKSKKSRFKLPKFNFSGSKVQTPEVDVKGKKPDIDITGPKVDINAPDVEVQGKVKGSKFKMPFLSISSPKVSMPDVELNLKSPKVKGDLDIAGPNLEGDFKGPKVDIKAPEVNLNAPDVDVHGPDWNLKMPKMKMPKFSVSGLKAEGPDVAVDLPKGDINIEGPSMNIEGPDLNVEGPEGGLKGPKFKMPDMNIKAPKISMPDIDLNLKGPKVKGDVDISLPKLEGDLKGPEVDIKGPKVDINAPDVDVHGPDWHLKMPKVKMPKFSMPGFKGEGPEVDVTLPKADIDISGPNVDVDVPDVNIEGPDAKLKGPKFKMPEMNIKAPKISMPDFDLNLKGPKMKGDVVVSLPKVEGDLKGPEVDIKGPKVDIDTPDINIEGSEGKFKGPKFKIPEMHLKAPKISMPDIDLNLKGPKVKGDVDVSLPKMEGDLKGPEVDIKGPKVDINAPDVDVQGPDWHLKMPKVKMPKFSMPGFKGEGPDVDVNLPKADLDVSGPKVDIDVPDVNIEGPEGKLKGPKFKMPEMNIKAPKISMPDIDLNLKGPKVKGDMDVSLPKVEGDMQVPDLDIKGPKVDINAPDVDVRGPDWHLKMPKIKMPKISMPGFKGEGPEVDVNLPKADLDVSGPKVDVDVPDVNIEGPDAKLKGPKFKMPEMNIKAPKISMPDFDLHLKGPKVKGDVDVSLPKMEGDLKAPEVDIKGPKVDIDAPDVDVHGPDWHLKMPKVKMPKFSMPGFKGEGPEVDVNLPKADIDVSGPKVDIDTPDIDIHGPEGKLKGPKFKMPDLHLKAPKISMPEVDLNLKGPKMKGDVDVSLPKVEGDLKGPEVDIKGPKVDIDVPDVDVQGPDWHLKMPKVKMPKFSMPGFKGEGPDVDVNLPKADLDVSGPKVDIDVPDVNIEGPDAKLKGPKFKMPEMNIKAPKISMPDFDLHLKGPKVKGDVDVSLPKVEGDLKGPEVDIKGPKVDIDAPDVDVHGPDWHLKMPKVKMPKFSMPGFKGEGPDVDVTLPKADIEISGPKVDIDAPDVSIEGPDAKLKGPKFKMPEMNIKAPKISMPDIDFNLKGPKVKGDVDVSLPKVEGDLKGPEIDIKGPSLDIDTPDVNIEGPEGKLKGPKFKMPEMNIKAPKISMPDFDLHLKGPKVKGDVDVSLPKVESDLKGPEVDIEGPEGKLKGPKFKMPDVHFKSPQISMSDIDLNLKGPKIKGDMDISVPKLEGDLKGPKVDVKGPKVGIDTPDIDIHGPEGKLKGPKFKMPDLHLKAPKISMPEVDLNLKGPKVKGDMDISLPKVEGDLKGPEVDIRDPKVDIDVPDVDVQGPDWHLKMPKVKMPKFSMPGFKGEGPDVDVNLPKADIDVSGPKVDVDVPDVNIEGPDAKLKGPKFKMPEMSIKAPKISMPDIDLNLKGPKVKGDVDVTLPKVEGDLKGPEADIKGPKVDINTPDVDVHGPDWHLKMPKVKMPKFSMPGFKGEGPDVDVSLPKADIDVSGPKVDVDIPDVNIEGPDAKLKGPKFKMPEINIKAPKISIPDVDLDLKGPKVKGDFDVSVPKVEGTLKGPEVDLKGPRLDFEGPDAKLSGPSLKMPSLEISAPKVTAPDVDLHLKAPKIGFSGPKLEGGEVDLKGPKVEAPSLDVHMDSPDINIEGPDVKIPKFKKPKFGFGAKSPKADIKSPSLDVTVPEAELNLETPEISVGGKGKKSKFKMPKIHMSGPKIKAKKQGFDLNVPGGEIDASLKAPDVDVNIAGPDAALKVDVKSPKTKKTMFGKMYFPDVEFDIKSPKFKAEAPLPSPKLEGELQAPDLELSLPAIHVEGLDIKAKAPKVKMPDVDISVPKIEGDLKGPKVQANLGAPDINIEGLDAKVKTPSFGISAPQVSIPDVNVNLKGPKIKGDVPSVGLEGPDVDLQGPEAKIKFPKFSMPKIGIPGVKMEGGGAEVHAQLPSLEGDLRGPDVKLEGPDVSLKGPGVDLPSVNLSMPKVSGPDLDLNLKGPSLKGDLDASVPSMKVHAPGLNLSGVGGKMQVGGDGVKVPGIDATTKLNVGAPDVTLRGPSLQGDLAVSGDIKCPKVSVGAPDLSLEASEGSIKLPKMKLPQFGISTPGSDLHVNAKGPQVSGELKGPGVDVNLKGPRISAPNVDFNLEGPKVKGSLGATGEIKGPTVGGGLPGIGVQGLEGNLQMPGIKSSGCDVNLPGVNVKLPTGQISGPEIKGGLKGSEVGFHGAAPDISVKGPAFNMASPESDFGINLKGPKIKGGADVSGGVSAPDISLGEGHLSVKGSGGEWKGPQVSSALNLDTSKFAGGLHFSGPKVEGGVKGGQIGLQAPGLSVSGPQGHLESGSGKVTFPKMKIPKFTFSGRELVGREMGVDVHFPKAEASIQAGAGDGEWEESEVKLKKSKIKMPKFNFSKPKGKGGVTGSPEASISGSKGDLKSSKASLGSLEGEAEAEASSPKGKFSLFKSKKPRHRSNSFSDEREFSGPSTPTGTLEFEGGEVSLEGGKVKGKHGKLKFGTFGGLGSKSKGHYEVTGSDDETGKLQGSGVSLASKKSRLSSSSSNDSGNKVGIQLPEVELSVSTKKE

SEQ ID NO: 17 - DNA, 324 bp, Homo sapiens
  source 1..324: mol_type = genomic DNA
cacctgaagatgcccaaggtgaaaatgcccaagttcagcatgcctggcttcaaaggagagggcccagatgtggatgtgaacctgcccaaggctgaccttgatgtctcaggacccaaggtggacattgatgttccagatgtgaatatcgaaggcccagagggaaagttgaaaggtcccaaattcaagatgcctgagatgaacatcaaagcccccaagatctccatgcctgacattgatcttaacctgaaaggacccaaagtgaagggtgatatggatgtgtctctgccaaaagtggaaggtgacatgcaagttcctgacttggat

SEQ ID NO: 18 - DNA, 384 bp, Homo sapiens
  source 1..384: mol_type = genomic DNA
cacctaaaaatgcccaaagtgaaaatgcccaagttcagcatgcctggcttcaaaggagagggcccagatgtggatgtgaacctgcccaaggctgacattgatgtctcaggacccaaagtggacgttgatgttcctgatgtgaatatcgaaggtccagatgcgaaactaaagggccccaagttcaagatgcctgagatgagcatcaaagcccccaagatctccatgcctgatattgacttaaacctgaaaggacccaaagtgaagggcgatgtggatgttacccttcctaaagtggaaggtgacctcaagggcccagaagctgacatcaagggcccaaaagtggacatcaacacccctgatgtggatgttcatggcccagactgg

SEQ ID NO: 19 - DNA, 9835 bp, synthetic construct
  source 1..9835: mol_type = other DNA
cctgcaggcagctgcgcgctcgctcgctcactgaggccgcccgggcaaagcccgggcgtcgggcgacctttggtcgcccggcctcagtgagcgagcgagcgcgcagagagggagtggccaactccatcactaggggttccttctagacaactttgtatagaaaagttgcgttacataacttacggtaaatggcccgcctggctgaccgcccaacgacccccgcccattgacgtcaatagtaacgccaatagggactttccattgacgtcaatgggtggagtatttacggtaaactgcccacttggcagtacatcaagtgtatcatatgccaagtacgccccctattgacgtcaatgacggtaaatggcccgcctggcattgtgcccagtacatgaccttatgggactttcctacttggcagtacatctacgtattagtcatcgctattaccatggtcgaggtgagccccacgttctgcttcactctccccatctcccccccctccccacccccaattttgtatttatttattttttaattattttgtgcagcgatgggggcggggggggggggggggcgcgcgccaggcggggcggggcggggcgaggggcggggcggggcgaggcggagaggtgcggcggcagccaatcagagcggcgcgctccgaaagtttccttttatggcgaggcggcggcggcggcggccctataaaaagcgaagcgcgcggcgggcgggagtcgctgcgcgctgccttcgccccgtgccccgctccgccgccgcctcgcgccgcccgccccggctctgactgaccgcgttactcccacaggtgagcgggcgggacggcccttctcctccgggctgtaattagctgagcaagaggtaagggtttaagggatggttggttggtggggtattaatgtttaattacctggagcacctgcctgaaatcactttttttcaggttggcaagtttgtacaaaaaagcaggctgccaccatggactacaaagaccatgacggtgattataaagatcatgacatcgactacaaggatgacgatgacaaggagaaggaggagacaacccgggagctgctgctgcccaactggcagggtagtggctcccacgggctgaccatcgcccagagggacgacggcgtctttgtgcaggaggtgacgcagaactcccctgcggcccgcactggggtggtcaaggagggggaccagattgtgggtgccaccatctactttgacaacctgcagtcgggtgaggtgacccagctgctgaacaccatggggcaccacacggtgggcctgaagctgcaccgcaagggggaccgctctcccgagcctggccagacctggacccgtgaagtcttcagctcctgcagctctgaagtggttctgagcggggatgatgaggagtaccagcgcatctacaccacgaagatcaagccacggctgaagtcggaagatggagtggaaggagacctcggggagacccagagccgtaccatcacagtgaccagaagggtcacggcctacactgtggatgtgactggccgggaaggagccaaggacatagacatcagtagccctgaattcaagatcaagattccaagacatgaactgactgaaatctccaatgtggatgtggagacccagtctgggaagaccgtgatcagactgccctcgggctcgggggcagcctctccgacaggctctgctgtggatatccgagcaggggccatttctgcttcaggaccagagctccaaggtgctggccactcgaagctccaggtcaccatgcctgggataaaggtgggaggctcaggtgtcaatgtcaatgcaaagggcttggacttgggtggcagaggaggggtccaagttccagcagtggacatttcatcttctcttgggggtagggcagtagaggtacagggcccatctctggagagtggtgatcatggcaaaattaaatttcccaccatgaaagtgccgaaatttggtgtctcaacagggcgtgagggccagacaccaaaggcagggctgagggtttctgcacctgaagtctctgtggggcacaagggcggcaagccaggcttgactatccaagcccctcagctggaagtcagtgtgccctctgccaatattgagggccttgaggggaagctgaagggcccccaaatcactgggccatcacttgagggtgacctaggcctgaaaggtgccaagccacaggggcacattggggtggatgcctctgctccccaaattgggggtagcatcactggccccagtgtggaagttcaggcccctgacattgatgttcaggggcctgggagcaaactgaatgtgcccaagatgaaagtccccaagttctctgtatcaggtgcaaagggagaggaaactgggattgatgtgacactgcctacaggtgaagtgactgttcctggggtctctggggatgtcagcctgcctgagattgctactggtgggctggaaggaaagatgaaaggtactaaagtgaagactcctgaaatgattattcagaaacctaaaatctccatgcaggatgtggatctgagccttgggtctcctaaactgaaaggagatattaaggtttctgctcctggggtgcaaggtgatgttaaaggccctcaagtggcacttaaaggctccagagtggacatagagacaccaaacctagagggaaccttgacaggccctaggcttggcagtccttccgggaaaaccggaacctgtaggatctctatgtcagaagtagacttaaatgtggccgcacctaaagtgaaagggggtgtagatgtcacactccccagagtagaagggaaagtcaaagtccctgaagttgatgtcagaggccccaaagtggatgtcagtgccccagatgtcgaagcgcatggcccagaatggaacctgaaaatgcccaagatgaaaatgcccacgttcagcactccaggagccaaaggggaaggtccagatgttcatatgactctacccaaaggagatatcagtatttcagggcccaaggtcaatgtggaagccccagatgtcaacttggagggtctggggggaaaacacctgaagatgcccaaggtgaaaatgcccaagttcagcatgcctggcttcaaaggagagggcccagatgtggatgtgaacctgcccaaggctgaccttgatgtctcaggacccaaggtggacattgatgttccagatgtgaatatcgaaggcccagagggaaagttgaaaggtcccaaattcaagatgcctgagatgaacatcaaagcccccaagatctccatgcctgacattgatcttaacctgaaaggacccaaagtgaagggtgatatggatgtgtctctgccaaaagtggaaggtgacatgcaagttcctgacttggatattaaaggccccaaagtggatattaatgccccagatgtggatgttcgaggcccagactggcacctaaaaatgcccaaagtgaaaatgcccaagttcagcatgcctggcttcaaaggagagggcccagatgtggatgtgaacctgcccaaggctgacattgatgtctcaggacccaaagtggacgttgatgttcctgatgtgaatatcgaaggtccagatgcgaaactaaagggccccaagttcaagatgcctgagatgagcatcaaagcccccaagatctccatgcctgatattgacttaaacctgaaaggacccaaagtgaagggcgatgtggatgttacccttcctaaagtggaaggtgacctcaagggcccagaagctgacatcaagggcccaaaagtggacatcaacacccctgatgtggatgttcatggcccagactggaagatgccatcgctggagatatctgctcctaaagtaactgctcctgatgttgatttgcatctcaaggcaccaaaaattggattttcaggtccgaagttagaaggtggtgaagtggacctcaagggacccaaagttgaagctccaagcttagatgtacacatggacagcccagatattaacatcgaagggccagatgttaaaatccccaaatttaagaaacccaagtttggatttggggcaaaaagccccaaagctgacatcaagtcaccttcactggatgtcactgttcctgaggcagagctgaaccttgagactcctgaaattagtgttggtggcaagggcaagaaaagtaagtttaaaatgcctaaaattcatatgagtggtcctaagattaaggccaaaaaacagggatttgacctgaatgttcctgggggtgaaattgatgccagcctcaaggctccggatgtagatgtcaacatcgcagggccggatgctgcactcaaagtcgacgtgaaatcgcccaaaaccaagaaaacgatgtttggaaaaatgtacttcccagatgtagagtttgacattaaatcacctaaatttaaagctgaggcccctctccctagccccaaactggagggtgaactccaggcacctgatctggaactttctttgccagcgattcacgtcgaaggtcttgacatcaaggcgaaggctcccaaggtcaagatgccagatgtggacatctcagtgccaaaaatagagggtgacctgaaaggccccaaagtgcaggcaaacttgggtgcacctgacatcaacatcgaaggcctagatgctaaagtcaaaacaccgtccttcggcatttctgcccctcaagtctccatccctgatgtgaatgtaaacttgaaaggaccaaagataaagggtgatgtccccagcgtgggactggaaggaccagatgtagatctgcaaggtccagaagcaaaaattaagttccccaagttttccatgcccaagatcggcatcccaggtgtgaaaatggagggtgggggagccgaggtccatgcccagctaccctctcttgaaggagacttgagaggaccagatgttaagctcgaagggcccgatgtttctctaaaggggccaggagtagacttgccttcagtgaacctctctatgccaaaagtctctgggcctgaccttgatctgaacttgaaaggaccaagtttgaagggagacctggatgcatctgttcccagcatgaaggtgcatgctccagggctcaacctcagtggtgtcggtggcaaaatgcaggtgggaggagacggtgtgaaagtgccagggatcgatgccacaacaaagcttaacgttggggcaccagatgtgacactgaggggaccaagcctgcagggagatctggctgtctctggtgacatcaaatgccctaaagtatccgtaggagctcctgatctaagcttggaggcatccgaaggcagcattaaacttcccaaaatgaagctgccccaatttggcatctctactccggggtccgacttgcacgtcaatgccaaggggccacaggtttctggcgaactgaaggggccaggtgtggatgtgaacctgaaagggcctcggatttcagcaccgaatgtggactttaacttggaaggaccaaaagtgaaagggagccttggggccactggtgagatcaaaggccccactgtcggaggaggtcttccaggcattggtgttcaaggcctagaaggaaacctccagatgcctggaattaagtcctctggatgtgatgtgaacctgccaggcgtgaatgtgaaactcccaactgggcagatttctgggcctgaaatcaaaggtggtctgaaaggttcagaagtaggtttccatggggctgctcctgatatcagtgtgaaggggcctgcctttaatatggcatctcctgagtcagattttggcatcaacttgaagggcccaaaaatcaaaggaggtgcggatgtttcagggggtgtcagtgccccagacatcagccttggtgaagggcatttgagtgttaaaggttccgggggtgagtggaagggaccccaagtctcctctgctctcaacttggacacatctaagtttgctgggggccttcatttctcaggaccaaaggtggaaggaggtgtgaaaggaggtcagattggactccaggctcctgggctgagtgtgtctgggcctcaaggtcacttggaaagtggatctggaaaagtaacattccctaaaatgaagatccccaaatttaccttctctggccgtgagctggttggcagagaaatgggggtggatgttcacttccctaaagcagaggccagcatccaagctggtgctggagacggcgagtgggaagagtctgaagtcaaactgaaaaagtccaagatcaaaatgcccaagtttaatttttccaaacctaaagggaaaggtggtgtcactggctcaccagaagcatcaatttctgggtccaaaggtgacctgaaaagttcaaaggccagcctgggctctctggaaggagaggcagaggccgaagcctcttcaccgaaaggcaaattctccttatttaaaagtaagaagccacggcaccgctcaaattcattcagtgatgaaagagagttctctggaccttccaccccgacggggacgctggagtttgaaggtggggaagtgtctctggaaggtgggaaagttaaagggaaacacgggaagctgaaattcggtacctttggtggattggggtcaaagagcaaaggtcattatgaggtgactgggagcgatgatgagacaggcaagttacaggggagtggggtgtccctggcctctaagaagtcccgactgtcctcctcttctagcaatgacagtgggaataaggttggcatccagcttcccgaggtggagctgtcagtttccacaaagaaagagtagacccagctttcttgtacaaagtgggaattcctagagctcgctgatcagcctcgactgtgccttctagttgccagccatctgttgtttgcccctcccccgtgccttccttgaccctggaaggtgccactcccactgtcctttcctaataaaatgaggaaattgcatcgcattgtctgagtaggtgtcattctattctggggggtggggtggggcaggacagcaagggggaggattgggaagagaatagcaggcatgctggggagggccgcaggaacccctagtgatggagttggccactccctctctgcgcgctcgctcgctcactgaggccgggcgaccaaaggtcgcccgacgcccgggctttgcccgggcggcctcagtgagcgagcgagcgcgcagctgcctgcaggggcgcctgatgcggtattttctccttacgcatctgtgcggtatttcacaccgcatacgtcaaagcaaccatagtacgcgccctgtagcggcgcattaagcgcggcgggggtggtggttacgcgcagcgtgaccgctacacttgccagcgccttagcgcccgctcctttcgctttcttcccttcctttctcgccacgttcgccggctttccccgtcaagctctaaatcgggggctccctttagggttccgatttagtgctttacggcacctcgaccccaaaaaacttgatttgggtgatggttcacgtagtgggccatcgccctgatagacggtttttcgccctttgacgttggagtccacgttctttaatagtggactcttgttccaaactggaacaacactcaactctatctcgggctattcttttgatttataagggattttgccgatttcggtctattggttaaaaaatgagctgatttaacaaaaatttaacgcgaattttaacaaaatattaacgtttacaattttatggtgcactctcagtacaatctgctctgatgccgcatagttaagccagccccgacacccgccaacacccgctgacgcgccctgacgggcttgtctgctcccggcatccgcttacagacaagctgtgaccgtctccgggagctgcatgtgtcagaggttttcaccgtcatcaccgaaacgcgcgagacgaaagggcctcgtgatacgcctatttttataggttaatgtcatgataataatggtttcttagacgtcaggtggcacttttcggggaaatgtgcgcggaacccctatttgtttatttttctaaatacattcaaatatgtatccgctcatgagacaataaccctgataaatgcttcaataatattgaaaaaggaagagtatgagtattcaacatttccgtgtcgcccttattcccttttttgcggcattttgccttcctgtttttgctcacccagaaacgctggtgaaagtaaaagatgctgaagatcagttgggtgcacgagtgggttacatcgaactggatctcaacagcggtaagatccttgagagttttcgccccgaagaacgttttccaatgatgagcacttttaaagttctgctatgtggcgcggtattatcccgtattgacgccgggcaagagcaactcggtcgccgcatacactattctcagaatgacttggttgagtactcaccagtcacagaaaagcatcttacggatggcatgacagtaagagaattatgcagtgctgccataaccatgagtgataacactgcggccaacttacttctgacaacgatcggaggaccgaaggagctaaccgcttttttgcacaacatgggggatcatgtaactcgccttgatcgttgggaaccggagctgaatgaagccataccaaacgacgagcgtgacaccacgatgcctgtagcaatggcaacaacgttgcgcaaactattaactggcgaactacttactctagcttcccggcaacaattaatagactggatggaggcggataaagttgcaggaccacttctgcgctcggcccttccggctggctggtttattgctgataaatctggagccggtgagcgtggaagccgcggtatcattgcagcactggggccagatggtaagccctcccgtatcgtagttatctacacgacggggagtcaggcaactatggatgaacgaaatagacagatcgctgagataggtgcctcactgattaagcattggtaactgtcagaccaagtttactcatatatactttagattgatttaaaacttcatttttaatttaaaaggatctaggtgaagatcctttttgataatctcatgaccaaaatcccttaacgtgagttttcgttccactgagcgtcagaccccgtagaaaagatcaaaggatcttcttgagatcctttttttctgcgcgtaatctgctgcttgcaaacaaaaaaaccaccgctaccagcggtggtttgtttgccggatcaagagctaccaactctttttccgaaggtaactggcttcagcagagcgcagataccaaatactgttcttctagtgtagccgtagttaggccaccacttcaagaactctgtagcaccgcctacatacctcgctctgctaatcctgttaccagtggctgctgccagtggcgataagtcgtgtcttaccgggttggactcaagacgatagttaccggataaggcgcagcggtcgggctgaacggggggttcgtgcacacagcccagcttggagcgaacgacctacaccgaactgagatacctacagcgtgagctatgagaaagcgccacgcttcccgaagggagaaaggcggacaggtatccggtaagcggcagggtcggaacaggagagcgcacgagggagcttccagggggaaacgcctggtatctttatagtcctgtcgggtttcgccacctctgacttgagcgtcgatttttgtgatgctcgtcaggggggcggagcctatggaaaaacgccagcaacgcggcctttttacggttcctggccttttgctggccttttgctcacatgt